European Patent Application EP 4 549 557 A1, published May 7, 2025. Title: Oncolytic Virus co-expressing CD55 and CD59. Applicant: SillaJen, Inc. Application KR. The sequence listing filed with the application follows.

SEQUENCE LISTING (44 sequences)

SEQ ID NO: 1 - protein, 352 aa, synthetic construct
  REGION 1..352: note = human CD55
MTVARPSVPAALPLLGELPRLLLLVLLCLPAVWGDCGLPPDVPNAQPALEGRTSFPEDTVITYKCEESFVKIPGEKDSVICLKGSQWSDIEEFCNRSCEVPTRLNSASLKQPYITQNYFPVGTVVEYECRPGYRREPSLSPKLTCLQNLKWSTAVEFCKKKSCPNPGEIRNGQIDVPGGILFGATISFSCNTGYKLFGSTSSFCLISGSSVQWSDPLPECREIYCPAPPQIDNGIIQGERDHYGYRQSVTYACNKGFTMIGEHSIYCTVNNDEGEWSGPPPECRGKSLTSKVPPTVQKPTTVNVPTTEVSPTSQKTTTKTTTPNAQATRSTPVSRTTKHFHETTPNKGSGTT

SEQ ID NO: 2 - DNA, 1055 bp, synthetic construct
  misc_feature 1..1055: note = human CD55
  source 1..1055: mol_type = other DNA
tgaccgtcgcgcggccgagcgtgcccgcggcgctgcccctcctcggggagctgccccggctgctgctgctggtgctgttgtgcctgccggccgtgtggggtgactgtggccttcccccagatgtacctaatgcccagccagctttggaaggccgtacaagttttcccgaggatactgtaataacgtacaaatgtgaagaaagctttgtgaaaattcctggcgagaaggactcagtgatctgccttaagggcagtcaatggtcagatattgaagagttctgcaatcgtagctgcgaggtgccaacaaggctaaattctgcatccctcaaacagccttatatcactcagaattattttccagtcggtactgttgtggaatatgagtgccgtccaggttacagaagagaaccttctctatcaccaaaactaacttgccttcagaatttaaaatggtccacagcagtcgaattttgtaaaaagaaatcatgccctaatccgggagaaatacgaaatggtcagattgatgtaccaggtggcatattatttggtgcaaccatctccttctcatgtaacacagggtacaaattatttggctcgacttctagtttttgtcttatttcaggcagctctgtccagtggagtgacccgttgccagagtgcagagaaatttattgtccagcaccaccacaaattgacaatggaataattcaaggggaacgtgaccattatggatatagacagtctgtaacgtatgcatgtaataaaggattcaccatgattggagagcactctatttattgtactgtgaataatgatgaaggagagtggagtggcccaccacctgaatgcagaggaaaatctctaacttccaaggtcccaccaacagttcagaaacctaccacagtaaatgttccaactacagaagtctcaccaacttctcagaaaaccaccacaaaaaccaccacaccaaatgctcaagcaacacggagtacacctgtttccaggacaaccaagcattttcatgaaacaaccccaaataaaggaagtggaaccact

SEQ ID NO: 3 - protein, 101 aa, synthetic construct
  REGION 1..101: note = human CD59
MGIQGGSVLFGLLLVLAVFCHSGHSLQCYNCPNPTADCKTAVNCSSDFDACLITKAGLQVYNKCWKFEHCNFNDVTTRLRENELTYYCCKKDLCNFNEQLE

SEQ ID NO: 4 - DNA, 303 bp, synthetic construct
  misc_feature 1..303: note = human CD59
  source 1..303: mol_type = other DNA
atgggaatccaaggagggtctgtcctgttcgggctgctgctcgtcctggctgtcttctgccattcaggtcatagcctgcagtgctacaactgtcctaacccaactgctgactgcaaaacagccgtcaattgttcatctgattttgatgcgtgtctcattaccaaagctgggttacaagtgtataacaagtgttggaagtttgagcattgcaatttcaacgacgtcacaacccgcttgagggaaaatgagctaacgtactactgctgcaagaaggacctgtgtaactttaacgaacagcttgaa

SEQ ID NO: 5 - DNA, 210 bp, synthetic construct
  misc_feature 1..210: note = pLEO160
  source 1..210: mol_type = other DNA
ttttattttttttttttggaatataaatatccggtaaaattgaaaaaatatacactaattagcgtctcgtttcagacgctagccggtaccccgggttcgaaatcgataagcttggatccggagagctcccaacctcgaggaattcggtaccccgggttcgaaatcgataagcttggatccggagagctcccaacctcgagctagctcgag

SEQ ID NO: 6 - DNA, 88 bp, synthetic construct
  misc_feature 1..88: note = pLEO38
  source 1..88: mol_type = other DNA
ttttattttttttttttggaatataaatatccggtaaaattgaaaaaatatacactaattagcgtctcgtttcagacgctagctcgag

SEQ ID NO: 7 - protein, 15 aa, synthetic construct
  REGION 1..15: note = (G4S)3
GGGGSGGGGSGGGGS

SEQ ID NO: 8 - DNA, 45 bp, synthetic construct
  misc_feature 1..45: note = (G4S)3
  source 1..45: mol_type = other DNA
ggtggtggcggttcaggcggaggtggctctggcggtggcggatcg

SEQ ID NO: 9 - protein, 40 aa, synthetic construct
  REGION 1..40: note = H3L transmembrane domain
LFDINVIGLIVILFIMFMLIFNVKSKLLWFLTGTFVTAFI

SEQ ID NO: 10 - DNA, 120 bp, synthetic construct
  misc_feature 1..120: note = H3L transmembrane domain
  source 1..120: mol_type = other DNA
ttgtttgatattaatgttataggtttgattgtaattttgtttattatgtttatgctcatctttaacgttaaatctaagctgttatggttccttacaggaacattcgttaccgcatttatc

SEQ ID NO: 11 - protein, 110 aa, synthetic construct
  REGION 1..110: note = A27L transmembrane domain
MDGTLFPGDDDLAIPATEFFSTKAAKKPEAKREAIVKADEDDNEETLKQRLTNLEKKITNVTTKFEQIEKCCKRNDEVLFRLENHAETLRAAMISLAKKIDVQTGRRPYE

SEQ ID NO: 12 - DNA, 330 bp, synthetic construct
  misc_feature 1..330: note = A27L transmembrane domain
  source 1..330: mol_type = other DNA
atggacggaactcttttccccggagatgacgatcttgcaattccagcaactgaatttttttctacaaaggctgctaaaaagccagaggctaaacgcgaagcaattgttaaagccgatgaagacgacaatgaggaaactctcaaacaacggctaactaatttggaaaaaaagattactaatgtaacaacaaagtttgaacaaatagaaaagtgttgtaaacgcaacgatgaagttctatttaggttggaaaatcacgctgaaactctaagagcggctatgatatctctggctaaaaagattgatgttcagactggacggcgtccatatgag

SEQ ID NO: 13 - protein, 29 aa, synthetic construct
  REGION 1..29: note = D8L transmembrane domain
FAIIAIVFVFILTAILFFMSRRYSREKQN

SEQ ID NO: 14 - DNA, 87 bp, synthetic construct
  misc_feature 1..87: note = D8L transmembrane domain
  source 1..87: mol_type = other DNA
ttcgcaattattgccatagtattcgtgtttatacttaccgctattctcttttttatgagtcgacgatattcgcgagaaaaacaaaac

SEQ ID NO: 15 - protein, 35 aa, synthetic construct
  REGION 1..35: note = A16L transmembrane domain
LGAAITLVVISVIFYFISIYSRPKIKTNDINVRRR

SEQ ID NO: 16 - DNA, 105 bp, synthetic construct
  misc_feature 1..105: note = A16L transmembrane domain
  source 1..105: mol_type = other DNA
ttgggcgcggccataacattggttgtaatatctgttattttctattttatatctatttattcgcgtactaaaattaaaacaaatgatataaatgttcgtagacga

SEQ ID NO: 17 - protein, 37 aa, synthetic construct
  REGION 1..37: note = F9L transmembrane domain
PWFLVGVAIILVIFTVAICSIRRNLALKYRYGTFLYV

SEQ ID NO: 18 - DNA, 111 bp, synthetic construct
  misc_feature 1..111: note = F9L transmembrane domain
  source 1..111: mol_type = other DNA
ccgtggtttctagtgggtgtagcaattattctagttatttttactgtagctatttgttctattagacgaaatctggctcttaaatacagatacggaacgtttttatacgtt

SEQ ID NO: 19 - protein, 21 aa, synthetic construct
  REGION 1..21: note = G9R transmembrane domain
LKLHLISLLSLLVIWILIVAI

SEQ ID NO: 20 - DNA, 63 bp, synthetic construct
  misc_feature 1..63: note = G9R transmembrane domain
  source 1..63: mol_type = other DNA
ctaaaattgcatttgatcagtttattatctctcttggtaatatggatactaattgtagctatt

SEQ ID NO: 21 - protein, 67 aa, synthetic construct
  REGION 1..67: note = L1R transmembrane domain
VQFYMIVIGVIILAALFMYYAKRMLFTSTNDKIKLILANKENVHWTTYMDTFFRTSPMVIATTDMQN

SEQ ID NO: 22 - DNA, 201 bp, synthetic construct
  misc_feature 1..201: note = L1R transmembrane domain
  source 1..201: mol_type = other DNA
gttcagttttatatgattgttatcggtgttataatattggcagcgttgtttatgtactatgccaagcgtatgttgttcacatccaccaatgataaaatcaaacttattttagccaataaggaaaacgtccattggactacttacatggacacattctttagaacttctccgatggttattgctaccacggatatgcaaaac

SEQ ID NO: 23 - protein, 21 aa, synthetic construct
  REGION 1..21: note = A9L transmembrane domain
FVVVRAIASMIMYLVLGIALL

SEQ ID NO: 24 - DNA, 63 bp, synthetic construct
  misc_feature 1..63: note = A9L transmembrane domain
  source 1..63: mol_type = other DNA
ttcgtcgttgttagagccattgcgagcatgataatgtatttagtattaggtatagcattgctg

SEQ ID NO: 25 - protein, 21 aa, synthetic construct
  REGION 1..21: note = A13L transmembrane domain
MIGILLLIGICVAVTVAILYA

SEQ ID NO: 26 - DNA, 63 bp, synthetic construct
  misc_feature 1..63: note = A13L transmembrane domain
  source 1..63: mol_type = other DNA
atgattggtattcttttgttgatcggtatttgcgtagcagttaccgtcgccatcctatatgcg

SEQ ID NO: 27 - protein, 21 aa, synthetic construct
  REGION 1..21: note = A21L transmembrane domain
MITLFLILCYFILIFNIIVPA

SEQ ID NO: 28 - DNA, 63 bp, synthetic construct
  misc_feature 1..63: note = A21L transmembrane domain
  source 1..63: mol_type = other DNA
atgataactttatttttaatcctatgttatttcattcttatttttaatattatagtacctgca

SEQ ID NO: 29 - protein, 21 aa, synthetic construct
  REGION 1..21: note = A28L transmembrane domain
MNSLSIFFIVVATAAVCLLFI

SEQ ID NO: 30 - DNA, 63 bp, synthetic construct
  misc_feature 1..63: note = A28L transmembrane domain
  source 1..63: mol_type = other DNA
atgaactctctatcaattttttttattgtggtagcgacggctgcggtgtgtttactttttatc

SEQ ID NO: 31 - protein, 17 aa, synthetic construct
  REGION 1..17: note = E10R transmembrane domain
AVWTIIFIVLSQAGLDG

SEQ ID NO: 32 - DNA, 51 bp, synthetic construct
  misc_feature 1..51: note = E10R transmembrane domain
  source 1..51: mol_type = other DNA
gccgtatggaccattatttttatagtactttcgcaagcgggtttagacggc

SEQ ID NO: 33 - protein, 21 aa, synthetic construct
  REGION 1..21: note = G3L transmembrane domain
MASLLYLILFLLFVCISYYFT

SEQ ID NO: 34 - DNA, 63 bp, synthetic construct
  misc_feature 1..63: note = G3L transmembrane domain
  source 1..63: mol_type = other DNA
atggcatctttattatatcttattttatttttgttattcgtatgtatttcttattattttaca

SEQ ID NO: 35 - protein, 21 aa, synthetic construct
  REGION 1..21: note = H2R transmembrane domain
TSTLIFFVIILAISALLLWFQ

SEQ ID NO: 36 - DNA, 63 bp, synthetic construct
  misc_feature 1..63: note = H2R transmembrane domain
  source 1..63: mol_type = other DNA
acatcaacacttatattctttgttattatattggcaattagtgcgctattactctggtttcag

SEQ ID NO: 37 - protein, 21 aa, synthetic construct
  REGION 1..21: note = I2L transmembrane domain
YWLIIIFFIVLILLLLIYLYL

SEQ ID NO: 38 - DNA, 63 bp, synthetic construct
  misc_feature 1..63: note = I2L transmembrane domain
  source 1..63: mol_type = other DNA
tattggttaattattattttttttatagttcttattctactactattgatatatttgtattta

SEQ ID NO: 39 - protein, 21 aa, synthetic construct
  REGION 1..21: note = J5L transmembrane domain
IIDIKWLPIGLLALAILILAF

SEQ ID NO: 40 - DNA, 63 bp, synthetic construct
  misc_feature 1..63: note = J5L transmembrane domain
  source 1..63: mol_type = other DNA
attatagatatcaaatggcttccgattggattactagcgttagctattttaatattagcattt

SEQ ID NO: 41 - protein, 21 aa, synthetic construct
  REGION 1..21: note = L5R transmembrane domain
IVLFEVFVVFILIYVFFRSEL

SEQ ID NO: 42 - DNA, 63 bp, synthetic construct
  misc_feature 1..63: note = L5R transmembrane domain
  source 1..63: mol_type = other DNA
atagttttatttgaagtattcgttgtattcattctaatatatgtattttttagatctgaatta

SEQ ID NO: 43 - protein, 21 aa, synthetic construct
  REGION 1..21: note = O3L transmembrane domain
LVVIMFFIAFAFCSWLSYSYL

SEQ ID NO: 44 - DNA, 63 bp, synthetic construct
  misc_feature 1..63: note = O3L transmembrane domain
  source 1..63: mol_type = other DNA
ctcgtcgtaattatgttttttatagcgtttgccttctgtagttggctatcatatagctatctg